European Patent Specification EP 3 769 090 B1, published November 15, 2023. Title: CRISPR/CAS DROPOUT SCREENING PLATFORM TO REVEAL GENETIC VULNERABILITIES ASSOCIATED WITH TAU AGGREGATION. Applicant: Regeneron Pharmaceuticals, Inc. The sequence listing filed with the application follows.

SEQUENCE LISTING (43 sequences)

SEQ ID NO: 1 - protein, 31 aa, Artificial Sequence
  Synthetic
QTAPVPMPDLKNVKSKIGSTENLKHQPGGGK

SEQ ID NO: 2 - protein, 31 aa, Artificial Sequence
  Synthetic
VQIINKKLDLSNVQSKCGSKDNIKHVPGGGS

SEQ ID NO: 3 - protein, 31 aa, Artificial Sequence
  Synthetic
VQIVYKPVDLSKVTSKCGSLGNIHHKPGGGQ

SEQ ID NO: 4 - protein, 32 aa, Artificial Sequence
  Synthetic
VEVKSEKLDFKDRVQSKIGSLDNITHVPGGGN

SEQ ID NO: 5 - DNA, 93 bp, Artificial Sequence
  Synthetic
cagacagcccccgtgcccatgccagacctgaagaatgtcaagtccaagatcggctccactgagaacctgaagcaccagccgggaggcgggaag

SEQ ID NO: 6 - DNA, 93 bp, Artificial Sequence
  Synthetic
gtgcagataattaataagaagctggatcttagcaacgtccagtccaagtgtggctcaaaggataatatcaaacacgtcccgggaggcggcagt

SEQ ID NO: 7 - DNA, 93 bp, Artificial Sequence
  Synthetic
gtgcaaatagtctacaaaccagttgacctgagcaaggtgacctccaagtgtggctcattaggcaacatccatcataaaccaggaggtggccag

SEQ ID NO: 8 - DNA, 96 bp, Artificial Sequence
  Synthetic
gtggaagtaaaatctgagaagcttgacttcaaggacagagtccagtcgaagattgggtccctggacaatatcacccacgtccctggcggaggaaat

SEQ ID NO: 9 - protein, 133 aa, Artificial Sequence
  Synthetic
LQTAPVPMPDLKNVKSKIGSTENLKHQPGGGKVQIINKKLDLSNVQSKCGSKDNIKHVPGGGSVQIVYKPVDLSKVTSKCGSLGNIHHKPGGGQVEVKSEKLDFKDRVQSKIGSLDNITHVPGGGNKKIETHK

SEQ ID NO: 10 - DNA, 399 bp, Artificial Sequence
  Synthetic
ctgcagacagcccccgtgcccatgccagacctgaagaatgtcaagtccaagatcggctccactgagaacctgaagcaccagccgggaggcgggaaggtgcagataattaataagaagctggatcttagcaacgtccagtccaagtgtggctcaaaggataatatcaaacacgtcccgggaggcggcagtgtgcaaatagtctacaaaccagttgacctgagcaaggtgacctccaagtgtggctcattaggcaacatccatcataaaccaggaggtggccaggtggaagtaaaatctgagaagcttgacttcaaggacagagtccagtcgaagattgggtccctggacaatatcacccacgtccctggcggaggaaataaaaagattgaaacccacaag

SEQ ID NO: 11 - protein, 133 aa, Artificial Sequence
  Synthetic
LQTAPVPMPDLKNVKSKIGSTENLKHQPGGGKVQIINKKLDLSNVQSKCGSKDNIKHVSGGGSVQIVYKPVDLSKVTSKCGSLGNIHHKPGGGQVEVKSEKLDFKDRVQSKIGSLDNITHVPGGGNKKIETHK

SEQ ID NO: 12 - DNA, 399 bp, Artificial Sequence
  Synthetic
ctgcagacagcccccgtgcccatgccagacctgaagaatgtcaagtccaagatcggctccactgagaacctgaagcaccagccgggaggcgggaaggtgcagataattaataagaagctggatcttagcaacgtccagtccaagtgtggctcaaaggataatatcaaacacgtctcgggaggcggcagtgtgcaaatagtctacaaaccagttgacctgagcaaggtgacctccaagtgtggctcattaggcaacatccatcataaaccaggaggtggccaggtggaagtaaaatctgagaagcttgacttcaaggacagagtccagtcgaagattgggtccctggacaatatcacccacgtccctggcggaggaaataaaaagattgaaacccacaag

SEQ ID NO: 13 - protein, 238 aa, Artificial Sequence
  Synthetic
VSKGEELFTGVVPILVELDGDVNGHKFSVSGEGEGDATYGKLTLKFICTTGKLPVPWPTLVTTLTWGVQCFSRYPDHMKQHDFFKSAMPEGYVQERTIFFKDDGNYKTRAEVKFEGDTLVNRIELKGIDFKEDGNILGHKLEYNYISHNVYITADKQKNGIKANFKIRHNIEDGSVQLADHYQQNTPIGDGPVLLPDNHYLSTQSALSKDPNEKRDHMVLLEFVTAAGITLGMDELYK

SEQ ID NO: 14 - DNA, 714 bp, Artificial Sequence
  Synthetic
gtgagcaagggcgaggagctgttcaccggggtggtgcccatcctggtcgagctggacggcgacgtaaacggccacaagttcagcgtgtccggcgagggcgagggcgatgccacctacggcaagctgaccctgaagttcatctgcaccaccggcaagctgcccgtgccctggcccaccctcgtgaccaccctgacctggggcgtgcagtgcttcagccgctaccccgaccacatgaagcagcacgacttcttcaagtccgccatgcccgaaggctacgtccaggagcgcaccatcttcttcaaggacgacggcaactacaagacccgcgccgaggtgaagttcgagggcgacaccctggtgaaccgcatcgagctgaagggcatcgacttcaaggaggacggcaacatcctggggcacaagctggagtacaactacatcagccacaacgtctatatcaccgccgacaagcagaagaacggcatcaaggccaacttcaagatccgccacaacatcgaggacggcagcgtgcagctcgccgaccactaccagcagaacacccccatcggcgacggccccgtgctgctgcccgacaaccactacctgagcacccagtccgccctgagcaaagaccccaacgagaagcgcgatcacatggtcctgctggagttcgtgaccgccgccgggatcactctcggcatggacgagctgtacaag

SEQ ID NO: 15 - protein, 236 aa, Artificial Sequence
  Synthetic
VSKGEELFTGVVPILVELDGDVNGHKFSVSGEGEGDATYGKLTLKFICTTGKLPVPWPTLVTTFGYGLQCFARYPDHMKQHDFFKSAMPEGYVQERTIFFKDDGNYKTRAEVKFEGDTLVNRIELKGIDFKEDGNILGHKLEYNYNSHNVYIMADKQKNGIKVNFKIRHNIEDGSVQLADHYQQNTPIGDGPVLLPDNHYLSYQSALSKDPNEKRDHMVLLEFVTAAGITLGMDEL

SEQ ID NO: 16 - DNA, 708 bp, Artificial Sequence
  Synthetic
gtgagcaagggcgaggagctgttcaccggggtggtgcccatcctggtcgagctggacggcgacgtaaacggccacaagttcagcgtgtccggcgagggcgagggcgatgccacctacggcaagctgaccctgaagttcatctgcaccaccggcaagctgcccgtgccctggcccaccctcgtgaccaccttcggctacggcctgcagtgcttcgcccgctaccccgaccacatgaagcagcacgacttcttcaagtccgccatgcccgaaggctacgtccaggagcgcaccatcttcttcaaggacgacggcaactacaagacccgcgccgaggtgaagttcgagggcgacaccctggtgaaccgcatcgagctgaagggcatcgacttcaaggaggacggcaacatcctggggcacaagctggagtacaactacaacagccacaacgtctatatcatggccgacaagcagaagaacggcatcaaggtgaacttcaagatccgccacaacatcgaggacggcagcgtgcagctcgccgaccactaccagcagaacacccccatcggcgacggccccgtgctgctgcccgacaaccactacctgagctaccagtccgccctgagcaaagaccccaacgagaagcgcgatcacatggtcctgctggagttcgtgaccgccgccgggatcactctcggcatggacgagctg

SEQ ID NO: 17 - RNA, 77 nt, Artificial Sequence
  Synthetic
guuuuagagcuagaaauagcaaguuaaaauaaggcuaguccguuaucaacuugaaaaaguggcaccgagucggugcu

SEQ ID NO: 18 - RNA, 82 nt, Artificial Sequence
  Synthetic
guuggaaccauucaaaacagcauagcaaguuaaaauaaggcuaguccguuaucaacuugaaaaaguggcaccgagucggugc

SEQ ID NO: 19 - RNA, 76 nt, Artificial Sequence
  Synthetic
guuuuagagcuagaaauagcaaguuaaaauaaggcuaguccguuaucaacuugaaaaaguggcaccgagucggugc

SEQ ID NO: 20 - RNA, 86 nt, Artificial Sequence
  Synthetic
guuuaagagcuaugcuggaaacagcauagcaaguuuaaauaaggcuaguccguuaucaacuugaaaaaguggcaccgagucggugc

SEQ ID NO: 21 - protein, 1392 aa, Artificial Sequence
  Synthetic
  MISC_FEATURE (1)..(1384): Cas9
  MISC_FEATURE (1385)..(1392): FLAG
MDKKYSIGLDIGTNSVGWAVITDEYKVPSKKFKVLGNTDRHSIKKNLIGALLFDSGETAEATRLKRTARRRYTRRKNRICYLQEIFSNEMAKVDDSFFHRLEESFLVEEDKKHERHPIFGNIVDEVAYHEKYPTIYHLRKKLVDSTDKADLRLIYLALAHMIKFRGHFLIEGDLNPDNSDVDKLFIQLVQTYNQLFEENPINASGVDAKAILSARLSKSRRLENLIAQLPGEKKNGLFGNLIALSLGLTPNFKSNFDLAEDAKLQLSKDTYDDDLDNLLAQIGDQYADLFLAAKNLSDAILLSDILRVNTEITKAPLSASMIKRYDEHHQDLTLLKALVRQQLPEKYKEIFFDQSKNGYAGYIDGGASQEEFYKFIKPILEKMDGTEELLVKLNREDLLRKQRTFDNGSIPHQIHLGELHAILRRQEDFYPFLKDNREKIEKILTFRIPYYVGPLARGNSRFAWMTRKSEETITPWNFEEVVDKGASAQSFIERMTNFDKNLPNEKVLPKHSLLYEYFTVYNELTKVKYVTEGMRKPAFLSGEQKKAIVDLLFKTNRKVTVKQLKEDYFKKIECFDSVEISGVEDRFNASLGTYHDLLKIIKDKDFLDNEENEDILEDIVLTLTLFEDREMIEERLKTYAHLFDDKVMKQLKRRRYTGWGRLSRKLINGIRDKQSGKTILDFLKSDGFANRNFMQLIHDDSLTFKEDIQKAQVSGQGDSLHEHIANLAGSPAIKKGILQTVKVVDELVKVMGRHKPENIVIEMARENQTTQKGQKNSRERMKRIEEGIKELGSQILKEHPVENTQLQNEKLYLYYLQNGRDMYVDQELDINRLSDYDVDHIVPQSFLKDDSIDNKVLTRSDKNRGKSDNVPSEEVVKKMKNYWRQLLNAKLITQRKFDNLTKAERGGLSELDKAGFIKRQLVETRQITKHVAQILDSRMNTKYDENDKLIREVKVITLKSKLVSDFRKDFQFYKVREINNYHHAHDAYLNAVVGTALIKKYPKLESEFVYGDYKVYDVRKMIAKSEQEIGKATAKYFFYSNIMNFFKTEITLANGEIRKRPLIETNGETGEIVWDKGRDFATVRKVLSMPQVNIVKKTEVQTGGFSKESILPKRNSDKLIARKKDWDPKKYGGFDSPTVAYSVLVVAKVEKGKSKKLKSVKELLGITIMERSSFEKNPIDFLEAKGYKEVKKDLIIKLPKYSLFELENGRKRMLASAGELQKGNELALPSKYVNFLYLASHYEKLKGSPEDNEQKQLFVEQHKHYLDEIIEQISEFSKRVILADANLDKVLSAYNKHRDKPIREQAENIIHLFTLTNLGAPAAFKYFDTTIDRKRYTSTKEVLDATLIHQSITGLYETRIDLSQLGGDKRPAATKKAGQAKKKKDYKDDDDK

SEQ ID NO: 22 - DNA, 4176 bp, Artificial Sequence
  Synthetic
  misc_feature (1)..(4152): Cas9
  misc_feature (4153)..(4176): FLAG
atggacaagaagtacagcatcggcctggacatcggcaccaactctgtgggctgggccgtgatcaccgacgagtacaaggtgcccagcaagaaattcaaggtgctgggcaacaccgaccggcacagcatcaagaagaacctgatcggagccctgctgttcgacagcggcgaaacagccgaggccacccggctgaagagaaccgccagaagaagatacaccagacggaagaaccggatctgctatctgcaagagatcttcagcaacgagatggccaaggtggacgacagcttcttccacagactggaagagtccttcctggtggaagaggataagaagcacgagcggcaccccatcttcggcaacatcgtggacgaggtggcctaccacgagaagtaccccaccatctaccacctgagaaagaaactggtggacagcaccgacaaggccgacctgcggctgatctatctggccctggcccacatgatcaagttccggggccacttcctgatcgagggcgacctgaaccccgacaacagcgacgtggacaagctgttcatccagctggtgcagacctacaaccagctgttcgaggaaaaccccatcaacgccagcggcgtggacgccaaggccatcctgtctgccagactgagcaagagcagacggctggaaaatctgatcgcccagctgcccggcgagaagaagaatggcctgttcggaaacctgattgccctgagcctgggcctgacccccaacttcaagagcaacttcgacctggccgaggatgccaaactgcagctgagcaaggacacctacgacgacgacctggacaacctgctggcccagatcggcgaccagtacgccgacctgtttctggccgccaagaacctgtccgacgccatcctgctgagcgacatcctgagagtgaacaccgagatcaccaaggcccccctgagcgcctctatgatcaagagatacgacgagcaccaccaggacctgaccctgctgaaagctctcgtgcggcagcagctgcctgagaagtacaaagagattttcttcgaccagagcaagaacggctacgccggctacattgacggcggagccagccaggaagagttctacaagttcatcaagcccatcctggaaaagatggacggcaccgaggaactgctcgtgaagctgaacagagaggacctgctgcggaagcagcggaccttcgacaacggcagcatcccccaccagatccacctgggagagctgcacgccattctgcggcggcaggaagatttttacccattcctgaaggacaaccgggaaaagatcgagaagatcctgaccttccgcatcccctactacgtgggccctctggccaggggaaacagcagattcgcctggatgaccagaaagagcgaggaaaccatcaccccctggaacttcgaggaagtggtggacaagggcgcttccgcccagagcttcatcgagcggatgaccaacttcgataagaacctgcccaacgagaaggtgctgcccaagcacagcctgctgtacgagtacttcaccgtgtataacgagctgaccaaagtgaaatacgtgaccgagggaatgagaaagcccgccttcctgagcggcgagcagaaaaaggccatcgtggacctgctgttcaagaccaaccggaaagtgaccgtgaagcagctgaaagaggactacttcaagaaaatcgagtgcttcgactccgtggaaatctccggcgtggaagatcggttcaacgcctccctgggcacataccacgatctgctgaaaattatcaaggacaaggacttcctggacaatgaggaaaacgaggacattctggaagatatcgtgctgaccctgacactgtttgaggacagagagatgatcgaggaacggctgaaaacctatgcccacctgttcgacgacaaagtgatgaagcagctgaagcggcggagatacaccggctggggcaggctgagccggaagctgatcaacggcatccgggacaagcagtccggcaagacaatcctggatttcctgaagtccgacggcttcgccaacagaaacttcatgcagctgatccacgacgacagcctgacctttaaagaggacatccagaaagcccaggtgtccggccagggcgatagcctgcacgagcacattgccaatctggccggcagccccgccattaagaagggcatcctgcagacagtgaaggtggtggacgagctcgtgaaagtgatgggccggcacaagcccgagaacatcgtgatcgaaatggccagagagaaccagaccacccagaagggacagaagaacagccgcgagagaatgaagcggatcgaagagggcatcaaagagctgggcagccagatcctgaaagaacaccccgtggaaaacacccagctgcagaacgagaagctgtacctgtactacctgcagaatgggcgggatatgtacgtggaccaggaactggacatcaaccggctgtccgactacgatgtggaccatatcgtgcctcagagctttctgaaggacgactccatcgacaacaaggtgctgaccagaagcgacaagaaccggggcaagagcgacaacgtgccctccgaagaggtcgtgaagaagatgaagaactactggcggcagctgctgaacgccaagctgattacccagagaaagttcgacaatctgaccaaggccgagagaggcggcctgagcgaactggataaggccggcttcatcaagagacagctggtggaaacccggcagatcacaaagcacgtggcacagatcctggactcccggatgaacactaagtacgacgagaatgacaagctgatccgggaagtgaaagtgatcaccctgaagtccaagctggtgtccgatttccggaaggatttccagttttacaaagtgcgcgagatcaacaactaccaccacgcccacgacgcctacctgaacgccgtcgtgggaaccgccctgatcaaaaagtaccctaagctggaaagcgagttcgtgtacggcgactacaaggtgtacgacgtgcggaagatgatcgccaagagcgagcaggaaatcggcaaggctaccgccaagtacttcttctacagcaacatcatgaactttttcaagaccgagattaccctggccaacggcgagatccggaagcggcctctgatcgagacaaacggcgaaaccggggagatcgtgtgggataagggccgggattttgccaccgtgcggaaagtgctgagcatgccccaagtgaatatcgtgaaaaagaccgaggtgcagacaggcggcttcagcaaagagtctatcctgcccaagaggaacagcgataagctgatcgccagaaagaaggactgggaccctaagaagtacggcggcttcgacagccccaccgtggcctattctgtgctggtggtggccaaagtggaaaagggcaagtccaagaaactgaagagtgtgaaagagctactggggatcaccatcatggaaagaagcagcttcgagaagaatcccatcgactttctggaagccaagggctacaaagaagtgaaaaaggacctgatcatcaagctgcctaagtactccctgttcgagctggaaaacggccggaagagaatgctggcctctgccggcgaactgcagaagggaaacgaactggccctgccctccaaatatgtgaacttcctgtacctggccagccactatgagaagctgaagggctcccccgaggataatgagcagaaacagctgtttgtggaacagcacaagcactacctggacgagatcatcgagcagatcagcgagttctccaagagagtgatcctggccgacgctaatctggacaaagtgctgtccgcctacaacaagcaccgggataagcccatcagagagcaggccgagaatatcatccacctgtttaccctgaccaatctgggagcccctgccgccttcaagtactttgacaccaccatcgaccggaagaggtacaccagcaccaaagaggtgctggacgccaccctgatccaccagagcatcaccggcctgtacgagacacggatcgacctgtctcagctgggaggcgacaagcgacctgccgccacaaagaaggctggacaggctaagaagaagaaagattacaaagacgatgacgataag

SEQ ID NO: 23 - RNA, 16 nt, Artificial Sequence
  Synthetic
guuuuagagcuaugcu

SEQ ID NO: 24 - RNA, 67 nt, Artificial Sequence
  Synthetic
agcauagcaaguuaaaauaaggcuaguccguuaucaacuugaaaaaguggcaccgagucggugcuuu

SEQ ID NO: 25 - DNA, 23 bp, Artificial Sequence
  Synthetic
  misc_feature (2)..(21): n = A, T, C, or G
gnnnnnnnnnnnnnnnnnnnngg

SEQ ID NO: 26 - DNA, 23 bp, Artificial Sequence
  Synthetic
  misc_feature (1)..(21): n = A, T, C, or G
nnnnnnnnnnnnnnnnnnnnngg

SEQ ID NO: 27 - DNA, 25 bp, Artificial Sequence
  Synthetic
  misc_feature (3)..(23): n = A, T, C, or G
ggnnnnnnnnnnnnnnnnnnnnngg

SEQ ID NO: 28 - RNA, 72 nt, Artificial Sequence
  Synthetic
aaacagcauagcaaguuaaaauaaggcuaguccguuaucaacuugaaaaaguggcaccgagucggugcuuuu

SEQ ID NO: 29 - RNA, 82 nt, Artificial Sequence; identical to SEQ ID NO: 18
  Synthetic

SEQ ID NO: 30 - RNA, 83 nt, Artificial Sequence
  Synthetic
guuuuagagcuagaaauagcaaguuaaaauaaggcuaguccguuaucaacuugaaaaaguggcaccgagucggugcuuuuuuu

SEQ ID NO: 31 - RNA, 80 nt, Artificial Sequence
  Synthetic
guuuuagagcuagaaauagcaaguuaaaauaaggcuaguccguuaucaacuugaaaaaguggcaccgagucggugcuuuu

SEQ ID NO: 32 - RNA, 92 nt, Artificial Sequence
  Synthetic
guuuaagagcuaugcuggaaacagcauagcaaguuuaaauaaggcuaguccguuaucaacuugaaaaaguggcaccgagucggugcuuuuuu

SEQ ID NO: 33 - RNA, 34 nt, Artificial Sequence
  Synthetic
ggccaacaugaggaucacccaugucugcagggcc

SEQ ID NO: 34 - RNA, 137 nt, Artificial Sequence
  Synthetic
guuuuagagcuaggccaacaugaggaucacccaugucugcagggccuagcaaguuaaaauaaggcuaguccguuaucaacuuggccaacaugaggaucacccaugucugcagggccaaguggcaccgagucggugcu

SEQ ID NO: 35 - RNA, 157 nt, Artificial Sequence
  Synthetic
  misc_feature (1)..(20): n is a, c, g, or u
nnnnnnnnnnnnnnnnnnnnguuuuagagcuaggccaacaugaggaucacccaugucugcagggccuagcaaguuaaaauaaggcuaguccguuaucaacuuggccaacaugaggaucacccaugucugcagggccaaguggcaccgagucggugcu

SEQ ID NO: 36 - protein, 1471 aa, Artificial Sequence
  Synthetic
  MISC_FEATURE (1)..(1384): dCas9
  MISC_FEATURE (1405)..(1409): NLS
  MISC_FEATURE (1410)..(1471): VP64
MKRPAATKKAGQAKKKKDKKYSIGLAIGTNSVGWAVITDEYKVPSKKFKVLGNTDRHSIKKNLIGALLFDSGETAEATRLKRTARRRYTRRKNRICYLQEIFSNEMAKVDDSFFHRLEESFLVEEDKKHERHPIFGNIVDEVAYHEKYPTIYHLRKKLVDSTDKADLRLIYLALAHMIKFRGHFLIEGDLNPDNSDVDKLFIQLVQTYNQLFEENPINASGVDAKAILSARLSKSRRLENLIAQLPGEKKNGLFGNLIALSLGLTPNFKSNFDLAEDAKLQLSKDTYDDDLDNLLAQIGDQYADLFLAAKNLSDAILLSDILRVNTEITKAPLSASMIKRYDEHHQDLTLLKALVRQQLPEKYKEIFFDQSKNGYAGYIDGGASQEEFYKFIKPILEKMDGTEELLVKLNREDLLRKQRTFDNGSIPHQIHLGELHAILRRQEDFYPFLKDNREKIEKILTFRIPYYVGPLARGNSRFAWMTRKSEETITPWNFEEVVDKGASAQSFIERMTNFDKNLPNEKVLPKHSLLYEYFTVYNELTKVKYVTEGMRKPAFLSGEQKKAIVDLLFKTNRKVTVKQLKEDYFKKIECFDSVEISGVEDRFNASLGTYHDLLKIIKDKDFLDNEENEDILEDIVLTLTLFEDREMIEERLKTYAHLFDDKVMKQLKRRRYTGWGRLSRKLINGIRDKQSGKTILDFLKSDGFANRNFMQLIHDDSLTFKEDIQKAQVSGQGDSLHEHIANLAGSPAIKKGILQTVKVVDELVKVMGRHKPENIVIEMARENQTTQKGQKNSRERMKRIEEGIKELGSQILKEHPVENTQLQNEKLYLYYLQNGRDMYVDQELDINRLSDYDVDHIVPQSFLKDDSIDNKVLTRSDKARGKSDNVPSEEVVKKMKNYWRQLLNAKLITQRKFDNLTKAERGGLSELDKAGFIKRQLVETRQITKHVAQILDSRMNTKYDENDKLIREVKVITLKSKLVSDFRKDFQFYKVREINNYHHAHDAYLNAVVGTALIKKYPKLESEFVYGDYKVYDVRKMIAKSEQEIGKATAKYFFYSNIMNFFKTEITLANGEIRKRPLIETNGETGEIVWDKGRDFATVRKVLSMPQVNIVKKTEVQTGGFSKESILPKRNSDKLIARKKDWDPKKYGGFDSPTVAYSVLVVAKVEKGKSKKLKSVKELLGITIMERSSFEKNPIDFLEAKGYKEVKKDLIIKLPKYSLFELENGRKRMLASAGELQKGNELALPSKYVNFLYLASHYEKLKGSPEDNEQKQLFVEQHKHYLDEIIEQISEFSKRVILADANLDKVLSAYNKHRDKPIREQAENIIHLFTLTNLGAPAAFKYFDTTIDRKRYTSTKEVLDATLIHQSITGLYETRIDLSQLGGDSAGGGGSGGGGSGGGGSGPKKKRKVAAAGSGRADALDDFDLDMLGSDALDDFDLDMLGSDALDDFDLDMLGSDALDDFDLDMLINCT

SEQ ID NO: 37 - protein, 473 aa, Artificial Sequence
  Synthetic
  MISC_FEATURE (1)..(130): MCP
  MISC_FEATURE (151)..(155): NLS
  MISC_FEATURE (161)..(341): P65
  MISC_FEATURE (350)..(473): HSF1
MASNFTQFVLVDNGGTGDVTVAPSNFANGVAEWISSNSRSQAYKVTCSVRQSSAQKRKYTIKVEVPKVATQTVGGVELPVAAWRSYLNMELTIPIFATNSDCELIVKAMQGLLKDGNPIPSAIAANSGIYSAGGGGSGGGGSGGGGSGPKKKRKVAAAGSPSGQISNQALALAPSSAPVLAQTMVPSSAMVPLAQPPAPAPVLTPGPPQSLSAPVPKSTQAGEGTLSEALLHLQFDADEDLGALLGNSTDPGVFTDLASVDNSEFQQLLNQGVSMSHSTAEPMLMEYPEAITRLVTGSQRPPDPAPTPLGTSGLPNGLSGDEDFSSIADMDFSALLSQISSSGQGGGGSGFSVDTSALLDLFSPSVTVPDMSLPDLDSSLASIQELLSPQEPPRPPEAENSSPDSGKQLVHYTAQPLFLLDPGSVDTGSNDLPVLFELGEGSYFSEGDGFAEDPTISLLTGSEPPKAKDPTVS

SEQ ID NO: 38 - DNA, 4413 bp, Artificial Sequence
  Synthetic
  misc_feature (1)..(4152): dCas9
  misc_feature (4213)..(4227): NLS
  misc_feature (4228)..(4413): VP64
atgaaaaggccggcggccacgaaaaaggccggccaggcaaaaaagaaaaaggacaagaagtacagcatcggcctggccatcggcaccaactctgtgggctgggccgtgatcaccgacgagtacaaggtgcccagcaagaaattcaaggtgctgggcaacaccgaccggcacagcatcaagaagaacctgatcggagccctgctgttcgacagcggcgaaacagccgaggccacccggctgaagagaaccgccagaagaagatacaccagacggaagaaccggatctgctatctgcaagagatcttcagcaacgagatggccaaggtggacgacagcttcttccacagactggaagagtccttcctggtggaagaggataagaagcacgagcggcaccccatcttcggcaacatcgtggacgaggtggcctaccacgagaagtaccccaccatctaccacctgagaaagaaactggtggacagcaccgacaaggccgacctgcggctgatctatctggccctggcccacatgatcaagttccggggccacttcctgatcgagggcgacctgaaccccgacaacagcgacgtggacaagctgttcatccagctggtgcagacctacaaccagctgttcgaggaaaaccccatcaacgccagcggcgtggacgccaaggccatcctgtctgccagactgagcaagagcagacggctggaaaatctgatcgcccagctgcccggcgagaagaagaatggcctgttcggcaacctgattgccctgagcctgggcctgacccccaacttcaagagcaacttcgacctggccgaggatgccaaactgcagctgagcaaggacacctacgacgacgacctggacaacctgctggcccagatcggcgaccagtacgccgacctgtttctggccgccaagaacctgtccgacgccatcctgctgagcgacatcctgagagtgaacaccgagatcaccaaggcccccctgagcgcctctatgatcaagagatacgacgagcaccaccaggacctgaccctgctgaaagctctcgtgcggcagcagctgcctgagaagtacaaagagattttcttcgaccagagcaagaacggctacgccggctacattgacggcggagccagccaggaagagttctacaagttcatcaagcccatcctggaaaagatggacggcaccgaggaactgctcgtgaagctgaacagagaggacctgctgcggaagcagcggaccttcgacaacggcagcatcccccaccagatccacctgggagagctgcacgccattctgcggcggcaggaagatttttacccattcctgaaggacaaccgggaaaagatcgagaagatcctgaccttccgcatcccctactacgtgggccctctggccaggggaaacagcagattcgcctggatgaccagaaagagcgaggaaaccatcaccccctggaacttcgaggaagtggtggacaagggcgcttccgcccagagcttcatcgagcggatgaccaacttcgataagaacctgcccaacgagaaggtgctgcccaagcacagcctgctgtacgagtacttcaccgtgtataacgagctgaccaaagtgaaatacgtgaccgagggaatgagaaagcccgccttcctgagcggcgagcagaaaaaggccatcgtggacctgctgttcaagaccaaccggaaagtgaccgtgaagcagctgaaagaggactacttcaagaaaatcgagtgcttcgactccgtggaaatctccggcgtggaagatcggttcaacgcctccctgggcacataccacgatctgctgaaaattatcaaggacaaggacttcctggacaatgaggaaaacgaggacattctggaagatatcgtgctgaccctgacactgtttgaggacagagagatgatcgaggaacggctgaaaacctatgcccacctgttcgacgacaaagtgatgaagcagctgaagcggcggagatacaccggctggggcaggctgagccggaagctgatcaacggcatccgggacaagcagtccggcaagacaatcctggatttcctgaagtccgacggcttcgccaacagaaacttcatgcagctgatccacgacgacagcctgacctttaaagaggacatccagaaagcccaggtgtccggccagggcgatagcctgcacgagcacattgccaatctggccggcagccccgccattaagaagggcatcctgcagacagtgaaggtggtggacgagctcgtgaaagtgatgggccggcacaagcccgagaacatcgtgatcgaaatggccagagagaaccagaccacccagaagggacagaagaacagccgcgagagaatgaagcggatcgaagagggcatcaaagagctgggcagccagatcctgaaagaacaccccgtggaaaacacccagctgcagaacgagaagctgtacctgtactacctgcagaatgggcgggatatgtacgtggaccaggaactggacatcaaccggctgtccgactacgatgtggaccacatcgtgcctcagagctttctgaaggacgactccatcgacaacaaggtgctgaccagaagcgacaaggcccggggcaagagcgacaacgtgccctccgaagaggtcgtgaagaagatgaagaactactggcggcagctgctgaacgccaagctgattacccagagaaagttcgacaatctgaccaaggccgagagaggcggcctgagcgaactggataaggccggcttcatcaagagacagctggtggaaacccggcagatcacaaagcacgtggcacagatcctggactcccggatgaacactaagtacgacgagaatgacaagctgatccgggaagtgaaagtgatcaccctgaagtccaagctggtgtccgatttccggaaggatttccagttttacaaagtgcgcgagatcaacaactaccaccacgcccacgacgcctacctgaacgccgtcgtgggaaccgccctgatcaaaaagtaccctaagctggaaagcgagttcgtgtacggcgactacaaggtgtacgacgtgcggaagatgatcgccaagagcgagcaggaaatcggcaaggctaccgccaagtacttcttctacagcaacatcatgaactttttcaagaccgagattaccctggccaacggcgagatccggaagcggcctctgatcgagacaaacggcgaaaccggggagatcgtgtgggataagggccgggattttgccaccgtgcggaaagtgctgagcatgccccaagtgaatatcgtgaaaaagaccgaggtgcagacaggcggcttcagcaaagagtctatcctgcccaagaggaacagcgataagctgatcgccagaaagaaggactgggaccctaagaagtacggcggcttcgacagccccaccgtggcctattctgtgctggtggtggccaaagtggaaaagggcaagtccaagaaactgaagagtgtgaaagagctgctggggatcaccatcatggaaagaagcagcttcgagaagaatcccatcgactttctggaagccaagggctacaaagaagtgaaaaaggacctgatcatcaagctgcctaagtactccctgttcgagctggaaaacggccggaagagaatgctggcctctgccggcgaactgcagaagggaaacgaactggccctgccctccaaatatgtgaacttcctgtacctggccagccactatgagaagctgaagggctcccccgaggataatgagcagaaacagctgtttgtggaacagcacaagcactacctggacgagatcatcgagcagatcagcgagttctccaagagagtgatcctggccgacgctaatctggacaaagtgctgtccgcctacaacaagcaccgggataagcccatcagagagcaggccgagaatatcatccacctgtttaccctgaccaatctgggagcccctgccgccttcaagtactttgacaccaccatcgaccggaagaggtacaccagcaccaaagaggtgctggacgccaccctgatccaccagagcatcaccggcctgtacgagacacggatcgacctgtctcagctgggaggcgacagcgctggaggaggtggaagcggaggaggaggaagcggaggaggaggtagcggacctaagaaaaagaggaaggtggcggccgctggatccggacgggctgacgcattggacgattttgatctggatatgctgggaagtgacgccctcgatgattttgaccttgacatgcttggttcggatgcccttgatgactttgacctcgacatgctcggcagtgacgcccttgatgatttcgacctggacatgctgattaactgtaca

SEQ ID NO: 39 - DNA, 1419 bp, Artificial Sequence
  Synthetic
  misc_feature (1)..(390): MCP
  misc_feature (451)..(465): NLS
  misc_feature (481)..(1023): P65
  misc_feature (1048)..(1419): HSF1
atggcttcaaactttactcagttcgtgctcgtggacaatggtgggacaggggatgtgacagtggctccttctaatttcgctaatggggtggcagagtggatcagctccaactcacggagccaggcctacaaggtgacatgcagcgtcaggcagtctagtgcccagaagagaaagtataccatcaaggtggaggtccccaaagtggctacccagacagtgggcggagtcgaactgcctgtcgccgcttggaggtcctacctgaacatggagctcactatcccaattttcgctaccaattctgactgtgaactcatcgtgaaggcaatgcaggggctcctcaaagacggtaatcctatcccttccgccatcgccgctaactcaggtatctacagcgctggaggaggtggaagcggaggaggaggaagcggaggaggaggtagcggacctaagaaaaagaggaaggtggcggccgctggatccccttcagggcagatcagcaaccaggccctggctctggcccctagctccgctccagtgctggcccagactatggtgccctctagtgctatggtgcctctggcccagccacctgctccagcccctgtgctgaccccaggaccaccccagtcactgagcgctccagtgcccaagtctacacaggccggcgaggggactctgagtgaagctctgctgcacctgcagttcgacgctgatgaggacctgggagctctgctggggaacagcaccgatcccggagtgttcacagatctggcctccgtggacaactctgagtttcagcagctgctgaatcagggcgtgtccatgtctcatagtacagccgaaccaatgctgatggagtaccccgaagccattacccggctggtgaccggcagccagcggccccccgaccccgctccaactcccctgggaaccagcggcctgcctaatgggctgtccggagatgaagacttctcaagcatcgctgatatggactttagtgccctgctgtcacagatttcctctagtgggcagggaggaggtggaagcggcttcagcgtggacaccagtgccctgctggacctgttcagcccctcggtgaccgtgcccgacatgagcctgcctgaccttgacagcagcctggccagtatccaagagctcctgtctccccaggagccccccaggcctcccgaggcagagaacagcagcccggattcagggaagcagctggtgcactacacagcgcagccgctgttcctgctggaccccggctccgtggacaccgggagcaacgacctgccggtgctgtttgagctgggagagggctcctacttctccgaaggggacggcttcgccgaggaccccaccatctccctgctgacaggctcggagcctcccaaagccaaggaccccactgtctcc

SEQ ID NO: 40 - protein, 130 aa, Artificial Sequence
  Synthetic
MASNFTQFVLVDNGGTGDVTVAPSNFANGVAEWISSNSRSQAYKVTCSVRQSSAQKRKYTIKVEVPKVATQTVGGVELPVAAWRSYLNMELTIPIFATNSDCELIVKAMQGLLKDGNPIPSAIAANSGIY

SEQ ID NO: 41 - DNA, 390 bp, Artificial Sequence
  Synthetic
atggcttcaaactttactcagttcgtgctcgtggacaatggtgggacaggggatgtgacagtggctccttctaatttcgctaatggggtggcagagtggatcagctccaactcacggagccaggcctacaaggtgacatgcagcgtcaggcagtctagtgcccagaagagaaagtataccatcaaggtggaggtccccaaagtggctacccagacagtgggcggagtcgaactgcctgtcgccgcttggaggtcctacctgaacatggagctcactatcccaattttcgctaccaattctgactgtgaactcatcgtgaaggcaatgcaggggctcctcaaagacggtaatcctatcccttccgccatcgccgctaactcaggtatctac

SEQ ID NO: 42 - DNA, 6673 bp, Artificial Sequence
  Synthetic
gtgcccgtcagtgggcagagcgcacatcgcccacagtccccgagaagttggggggaggggtcggcaattgaaccggtgcctagagaaggtggcgcggggtaaactgggaaagtgatgtcgtgtactggctccgcctttttcccgagggtgggggagaaccgtatataagtgcagtagtcgccgtgaacgttctttttcgcaacgggtttgccgccagaacacaggtaagtgccgtgtgtggttcccgcgggcctggcctctttacgggttatggcccttgcgtgccttgaattacttccacctggctgcagtacgtgattcttgatcccgagcttcgggttggaagtgggtgggagagttcgaggccttgcgcttaaggagccccttcgcctcgtgcttgagttgaggcctggcctgggcgctggggccgccgcgtgcgaatctggtggcaccttcgcgcctgtctcgctgctttcgataagtctctagccatttaaaatttttgatgacctgctgcgacgctttttttctggcaagatagtcttgtaaatgcgggccaagatctgcacactggtatttcggtttttggggccgcgggcggcgacggggcccgtgcgtcccagcgcacatgttcggcgaggcggggcctgcgagcgcggccaccgagaatcggacgggggtagtctcaagctggccggcctgctctggtgcctggcctcgcgccgccgtgtatcgccccgccctgggcggcaaggctggcccggtcggcaccagttgcgtgagcggaaagatggccgcttcccggccctgctgcagggagctcaaaatggaggacgcggcgctcgggagagcgggcgggtgagtcacccacacaaaggaaaagggcctttccgtcctcagccgtcgcttcatgtgactccacggagtaccgggcgccgtccaggcacctcgattagttctcgagcttttggagtacgtcgtctttaggttggggggaggggttttatgcgatggagtttccccacactgagtgggtggagactgaagttaggccagcttggcacttgatgtaattctccttggaatttgccctttttgagtttggatcttggttcattctcaagcctcagacagtggttcaaagtttttttcttccatttcaggtgtcgtgacgtacggccaccatgaaaaggccggcggccacgaaaaaggccggccaggcaaaaaagaaaaaggacaagaagtacagcatcggcctggccatcggcaccaactctgtgggctgggccgtgatcaccgacgagtacaaggtgcccagcaagaaattcaaggtgctgggcaacaccgaccggcacagcatcaagaagaacctgatcggagccctgctgttcgacagcggcgaaacagccgaggccacccggctgaagagaaccgccagaagaagatacaccagacggaagaaccggatctgctatctgcaagagatcttcagcaacgagatggccaaggtggacgacagcttcttccacagactggaagagtccttcctggtggaagaggataagaagcacgagcggcaccccatcttcggcaacatcgtggacgaggtggcctaccacgagaagtaccccaccatctaccacctgagaaagaaactggtggacagcaccgacaaggccgacctgcggctgatctatctggccctggcccacatgatcaagttccggggccacttcctgatcgagggcgacctgaaccccgacaacagcgacgtggacaagctgttcatccagctggtgcagacctacaaccagctgttcgaggaaaaccccatcaacgccagcggcgtggacgccaaggccatcctgtctgccagactgagcaagagcagacggctggaaaatctgatcgcccagctgcccggcgagaagaagaatggcctgttcggcaacctgattgccctgagcctgggcctgacccccaacttcaagagcaacttcgacctggccgaggatgccaaactgcagctgagcaaggacacctacgacgacgacctggacaacctgctggcccagatcggcgaccagtacgccgacctgtttctggccgccaagaacctgtccgacgccatcctgctgagcgacatcctgagagtgaacaccgagatcaccaaggcccccctgagcgcctctatgatcaagagatacgacgagcaccaccaggacctgaccctgctgaaagctctcgtgcggcagcagctgcctgagaagtacaaagagattttcttcgaccagagcaagaacggctacgccggctacattgacggcggagccagccaggaagagttctacaagttcatcaagcccatcctggaaaagatggacggcaccgaggaactgctcgtgaagctgaacagagaggacctgctgcggaagcagcggaccttcgacaacggcagcatcccccaccagatccacctgggagagctgcacgccattctgcggcggcaggaagatttttacccattcctgaaggacaaccgggaaaagatcgagaagatcctgaccttccgcatcccctactacgtgggccctctggccaggggaaacagcagattcgcctggatgaccagaaagagcgaggaaaccatcaccccctggaacttcgaggaagtggtggacaagggcgcttccgcccagagcttcatcgagcggatgaccaacttcgataagaacctgcccaacgagaaggtgctgcccaagcacagcctgctgtacgagtacttcaccgtgtataacgagctgaccaaagtgaaatacgtgaccgagggaatgagaaagcccgccttcctgagcggcgagcagaaaaaggccatcgtggacctgctgttcaagaccaaccggaaagtgaccgtgaagcagctgaaagaggactacttcaagaaaatcgagtgcttcgactccgtggaaatctccggcgtggaagatcggttcaacgcctccctgggcacataccacgatctgctgaaaattatcaaggacaaggacttcctggacaatgaggaaaacgaggacattctggaagatatcgtgctgaccctgacactgtttgaggacagagagatgatcgaggaacggctgaaaacctatgcccacctgttcgacgacaaagtgatgaagcagctgaagcggcggagatacaccggctggggcaggctgagccggaagctgatcaacggcatccgggacaagcagtccggcaagacaatcctggatttcctgaagtccgacggcttcgccaacagaaacttcatgcagctgatccacgacgacagcctgacctttaaagaggacatccagaaagcccaggtgtccggccagggcgatagcctgcacgagcacattgccaatctggccggcagccccgccattaagaagggcatcctgcagacagtgaaggtggtggacgagctcgtgaaagtgatgggccggcacaagcccgagaacatcgtgatcgaaatggccagagagaaccagaccacccagaagggacagaagaacagccgcgagagaatgaagcggatcgaagagggcatcaaagagctgggcagccagatcctgaaagaacaccccgtggaaaacacccagctgcagaacgagaagctgtacctgtactacctgcagaatgggcgggatatgtacgtggaccaggaactggacatcaaccggctgtccgactacgatgtggaccacatcgtgcctcagagctttctgaaggacgactccatcgacaacaaggtgctgaccagaagcgacaaggcccggggcaagagcgacaacgtgccctccgaagaggtcgtgaagaagatgaagaactactggcggcagctgctgaacgccaagctgattacccagagaaagttcgacaatctgaccaaggccgagagaggcggcctgagcgaactggataaggccggcttcatcaagagacagctggtggaaacccggcagatcacaaagcacgtggcacagatcctggactcccggatgaacactaagtacgacgagaatgacaagctgatccgggaagtgaaagtgatcaccctgaagtccaagctggtgtccgatttccggaaggatttccagttttacaaagtgcgcgagatcaacaactaccaccacgcccacgacgcctacctgaacgccgtcgtgggaaccgccctgatcaaaaagtaccctaagctggaaagcgagttcgtgtacggcgactacaaggtgtacgacgtgcggaagatgatcgccaagagcgagcaggaaatcggcaaggctaccgccaagtacttcttctacagcaacatcatgaactttttcaagaccgagattaccctggccaacggcgagatccggaagcggcctctgatcgagacaaacggcgaaaccggggagatcgtgtgggataagggccgggattttgccaccgtgcggaaagtgctgagcatgccccaagtgaatatcgtgaaaaagaccgaggtgcagacaggcggcttcagcaaagagtctatcctgcccaagaggaacagcgataagctgatcgccagaaagaaggactgggaccctaagaagtacggcggcttcgacagccccaccgtggcctattctgtgctggtggtggccaaagtggaaaagggcaagtccaagaaactgaagagtgtgaaagagctgctggggatcaccatcatggaaagaagcagcttcgagaagaatcccatcgactttctggaagccaagggctacaaagaagtgaaaaaggacctgatcatcaagctgcctaagtactccctgttcgagctggaaaacggccggaagagaatgctggcctctgccggcgaactgcagaagggaaacgaactggccctgccctccaaatatgtgaacttcctgtacctggccagccactatgagaagctgaagggctcccccgaggataatgagcagaaacagctgtttgtggaacagcacaagcactacctggacgagatcatcgagcagatcagcgagttctccaagagagtgatcctggccgacgctaatctggacaaagtgctgtccgcctacaacaagcaccgggataagcccatcagagagcaggccgagaatatcatccacctgtttaccctgaccaatctgggagcccctgccgccttcaagtactttgacaccaccatcgaccggaagaggtacaccagcaccaaagaggtgctggacgccaccctgatccaccagagcatcaccggcctgtacgagacacggatcgacctgtctcagctgggaggcgacagcgctggaggaggtggaagcggaggaggaggaagcggaggaggaggtagcggacctaagaaaaagaggaaggtggcggccgctggatccggacgggctgacgcattggacgattttgatctggatatgctgggaagtgacgccctcgatgattttgaccttgacatgcttggttcggatgcccttgatgactttgacctcgacatgctcggcagtgacgcccttgatgatttcgacctggacatgctgattaactgtacaggcagtggagagggcagaggaagtctgctaacatgcggtgacgtcgaggagaatcctggcccaatggccaagcctttgtctcaagaagaatccaccctcattgaaagagcaacggctacaatcaacagcatccccatctctgaagactacagcgtcgccagcgcagctctctctagcgacggccgcatcttcactggtgtcaatgtatatcattttactgggggaccttgtgcagaactcgtggtgctgggcactgctgctgctgcggcagctggcaacctgacttgtatcgtcgcgatcggaaatgagaacaggggcatcttgagcccctgcggacggtgccgacaggtgcttctcgatctgcatcctgggatcaaagccatagtgaaggacagtgatggacagccgacggcagttgggattcgtgaattgctgccctctggttatgtgtgggagggctaagaattcgatatcaagcttatcggtaatcaacctctggattacaaaatttgtgaaagattgactggtattcttaactatgttgctccttttacgctatgtggatacgctgctttaatgcctttgtatcatgctattgcttcccgtatggctttcattttctcctccttgtataaatcctggttgctgtctctttatgaggagttgtggcccgttgtcaggcaacgtggcgtggtgtgcactgtgtttgctgacgcaacccccactggttggggcattgccaccacctgtcagctcctttccgggactttcgctttccccctccctattgccacggcggaactcatcgccgcctgccttgcccgctgctggacaggggctcggctgttgggcactgacaattccgtggtgttgtcggggaaatcatcgtcctttccttggctgctcgcctgtgttgccacctggattctgcgcgggacgtccttctgctacgtcccttcggccctcaatccagcggaccttccttcccgcggcctgctgccggctctgcggcctcttccgcgtcttcgccttcgccctcagacgagtcggatctccctttgggccgcctccccgca

SEQ ID NO: 43 - DNA, 4324 bp, Artificial Sequence
  Synthetic
gtgcccgtcagtgggcagagcgcacatcgcccacagtccccgagaagttggggggaggggtcggcaattgaaccggtgcctagagaaggtggcgcggggtaaactgggaaagtgatgtcgtgtactggctccgcctttttcccgagggtgggggagaaccgtatataagtgcagtagtcgccgtgaacgttctttttcgcaacgggtttgccgccagaacacaggtaagtgccgtgtgtggttcccgcgggcctggcctctttacgggttatggcccttgcgtgccttgaattacttccacctggctgcagtacgtgattcttgatcccgagcttcgggttggaagtgggtgggagagttcgaggccttgcgcttaaggagccccttcgcctcgtgcttgagttgaggcctggcctgggcgctggggccgccgcgtgcgaatctggtggcaccttcgcgcctgtctcgctgctttcgataagtctctagccatttaaaatttttgatgacctgctgcgacgctttttttctggcaagatagtcttgtaaatgcgggccaagatctgcacactggtatttcggtttttggggccgcgggcggcgacggggcccgtgcgtcccagcgcacatgttcggcgaggcggggcctgcgagcgcggccaccgagaatcggacgggggtagtctcaagctggccggcctgctctggtgcctggcctcgcgccgccgtgtatcgccccgccctgggcggcaaggctggcccggtcggcaccagttgcgtgagcggaaagatggccgcttcccggccctgctgcagggagctcaaaatggaggacgcggcgctcgggagagcgggcgggtgagtcacccacacaaaggaaaagggcctttccgtcctcagccgtcgcttcatgtgactccacggagtaccgggcgccgtccaggcacctcgattagttctcgagcttttggagtacgtcgtctttaggttggggggaggggttttatgcgatggagtttccccacactgagtgggtggagactgaagttaggccagcttggcacttgatgtaattctccttggaatttgccctttttgagtttggatcttggttcattctcaagcctcagacagtggttcaaagtttttttcttccatttcaggtgtcgtgacgtacggccaccatggcttcaaactttactcagttcgtgctcgtggacaatggtgggacaggggatgtgacagtggctccttctaatttcgctaatggggtggcagagtggatcagctccaactcacggagccaggcctacaaggtgacatgcagcgtcaggcagtctagtgcccagaagagaaagtataccatcaaggtggaggtccccaaagtggctacccagacagtgggcggagtcgaactgcctgtcgccgcttggaggtcctacctgaacatggagctcactatcccaattttcgctaccaattctgactgtgaactcatcgtgaaggcaatgcaggggctcctcaaagacggtaatcctatcccttccgccatcgccgctaactcaggtatctacagcgctggaggaggtggaagcggaggaggaggaagcggaggaggaggtagcggacctaagaaaaagaggaaggtggcggccgctggatccccttcagggcagatcagcaaccaggccctggctctggcccctagctccgctccagtgctggcccagactatggtgccctctagtgctatggtgcctctggcccagccacctgctccagcccctgtgctgaccccaggaccaccccagtcactgagcgctccagtgcccaagtctacacaggccggcgaggggactctgagtgaagctctgctgcacctgcagttcgacgctgatgaggacctgggagctctgctggggaacagcaccgatcccggagtgttcacagatctggcctccgtggacaactctgagtttcagcagctgctgaatcagggcgtgtccatgtctcatagtacagccgaaccaatgctgatggagtaccccgaagccattacccggctggtgaccggcagccagcggccccccgaccccgctccaactcccctgggaaccagcggcctgcctaatgggctgtccggagatgaagacttctcaagcatcgctgatatggactttagtgccctgctgtcacagatttcctctagtgggcagggaggaggtggaagcggcttcagcgtggacaccagtgccctgctggacctgttcagcccctcggtgaccgtgcccgacatgagcctgcctgaccttgacagcagcctggccagtatccaagagctcctgtctccccaggagccccccaggcctcccgaggcagagaacagcagcccggattcagggaagcagctggtgcactacacagcgcagccgctgttcctgctggaccccggctccgtggacaccgggagcaacgacctgccggtgctgtttgagctgggagagggctcctacttctccgaaggggacggcttcgccgaggaccccaccatctccctgctgacaggctcggagcctcccaaagccaaggaccccactgtctcctgtacaggcagtggagagggcagaggaagtctgctaacatgcggtgacgtcgaggagaatcctggcccaaccatgaaaaagcctgaactcaccgctacctctgtcgagaagtttctgatcgaaaagttcgacagcgtctccgacctgatgcagctctccgagggcgaagaatctcgggctttcagcttcgatgtgggagggcgtggatatgtcctgcgggtgaatagctgcgccgatggtttctacaaagatcgctatgtttatcggcactttgcatccgccgctctccctattcccgaagtgcttgacattggggagttcagcgagagcctgacctattgcatctcccgccgtgcacagggtgtcaccttgcaagacctgcctgaaaccgaactgcccgctgttctccagcccgtcgccgaggccatggatgccatcgctgccgccgatcttagccagaccagcgggttcggcccattcggacctcaaggaatcggtcaatacactacatggcgcgatttcatctgcgctattgctgatccccatgtgtatcactggcaaactgtgatggacgacaccgtcagtgcctccgtcgcccaggctctcgatgagctgatgctttgggccgaggactgccccgaagtccggcacctcgtgcacgccgatttcggctccaacaatgtcctgaccgacaatggccgcataacagccgtcattgactggagcgaggccatgttcggggattcccaatacgaggtcgccaacatcttcttctggaggccctggttggcttgtatggagcagcagacccgctacttcgagcggaggcatcccgagcttgcaggatctcctcggctccgggcttatatgctccgcattggtcttgaccaactctatcagagcttggttgacggcaatttcgatgatgcagcttgggctcagggtcgctgcgacgcaatcgtccggtccggagccgggactgtcgggcgtacacaaatcgcccgcagaagcgctgccgtctggaccgatggctgtgtggaagtgctcgccgatagtggaaacagacgccccagcactcgtcctagggcaaaggatctgcagtaatgagaattcgatatcaagcttatcggtaatcaacctctggattacaaaatttgtgaaagattgactggtattcttaactatgttgctccttttacgctatgtggatacgctgctttaatgcctttgtatcatgctattgcttcccgtatggctttcattttctcctccttgtataaatcctggttgctgtctctttatgaggagttgtggcccgttgtcaggcaacgtggcgtggtgtgcactgtgtttgctgacgcaacccccactggttggggcattgccaccacctgtcagctcctttccgggactttcgctttccccctccctattgccacggcggaactcatcgccgcctgccttgcccgctgctggacaggggctcggctgttgggcactgacaattccgtggtgttgtcggggaaatcatcgtcctttccttggctgctcgcctgtgttgccacctggattctgcgcgggacgtccttctgctacgtcccttcggccctcaatccagcggaccttccttcccgcggcctgctgccggctctgcggcctcttccgcgtcttcgccttcgccctcagacgagtcggatctccctttgggccgcctccccgca